European Patent Application EP 4 190 347 A1, published June 7, 2023. Title: SCO-spondin-derived polypeptides for treating biological barriers dysfunction. Applicant: AXOLTIS PHARMA. The sequence listing filed with the application follows.

SEQUENCE LISTING (63 sequences)

SEQ ID NO: 1 - protein, 14 aa, artificial sequence
  Peptide compound
  MISC_FEATURE (1)..(1): Xaa  is absent or 1 to 6 amino acids
  MISC_FEATURE (4)..(4): Xaa  is 1 to 5 amino acids
  MISC_FEATURE (7)..(7): Xaa is 1 to 5 amino acids
  MISC_FEATURE (10)..(11): Xaa is 1 to 5 amino acids
  MISC_FEATURE (14)..(14): Xaa is  absent or is 1 to 6 amino acids
XWSXWSXCSXXCGX

SEQ ID NO: 2 - protein, 12 aa, Artificial sequence
  Peptide compound
  MISC_FEATURE (3)..(3): Xaa is 1 to 5 amino acids
  MISC_FEATURE (6)..(6): Xaa is 1 to 5 amino acids
  MISC_FEATURE (9)..(10): Xaa is 1 to 5 amino acids
WSXWSXCSXXCG

SEQ ID NO: 3 - protein, 12 aa, Artificial sequence
  Peptide compound
WSGWSSCSRSCG

SEQ ID NO: 4 - protein, 12 aa, Artificial sequence
  Peptide compound
WSSWSGCSRSCG

SEQ ID NO: 5 - protein, 12 aa, artificial sequence
  peptide compound
WSSWGSCSRSCG

SEQ ID NO: 6 - protein, 12 aa, artificial sequence
  peptide compound
WSSWGGCSRSCG

SEQ ID NO: 7 - protein, 12 aa, artificial sequence
  peptide compound
WSSWSSCSRSCG

SEQ ID NO: 8 - protein, 12 aa, artificial sequence
  peptide compound
WSGWSGCSRSCG

SEQ ID NO: 9 - protein, 12 aa, artificial sequence
  peptide compound
WSGWGSCSRSCG

SEQ ID NO: 10 - protein, 12 aa, artificial sequence
  peptide compound
WSGWGGCSRSCG

SEQ ID NO: 11 - protein, 12 aa, artificial sequence
  peptide compound
WSSWSSCSVSCG

SEQ ID NO: 12 - protein, 12 aa, artificial sequence
  peptide compound
WSSWSGCSVSCG

SEQ ID NO: 13 - protein, 12 aa, artificial sequence
  peptide compound
WSSWGSCSVSCG

SEQ ID NO: 14 - protein, 12 aa, artificial sequence
  peptide compound
WSSWGGCSVSCG

SEQ ID NO: 15 - protein, 12 aa, artificial sequence
  peptide compound
WSGWSSCSVSCG

SEQ ID NO: 16 - protein, 12 aa, artificial sequence
  peptide compound
WSGWSGCSVSCG

SEQ ID NO: 17 - protein, 12 aa, artificial sequence
  peptide compound
WSGWGSCSVSCG

SEQ ID NO: 18 - protein, 12 aa, artificial sequence
  peptide compound
WSGWGGCSVSCG

SEQ ID NO: 19 - protein, 12 aa, artificial sequence
  peptide compound
WSSWSSCSVTCG

SEQ ID NO: 20 - protein, 12 aa, artificial sequence
  peptide compound
WSSWSGCSVTCG

SEQ ID NO: 21 - protein, 12 aa, artificial sequence
  peptide compound
WSSWGSCSVTCG

SEQ ID NO: 22 - protein, 12 aa, artificial sequence
  peptide compound
WSSWGGCSVTCG

SEQ ID NO: 23 - protein, 12 aa, artificial sequence
  peptide compound
WSGWSSCSVTCG

SEQ ID NO: 24 - protein, 12 aa, Artificial Sequence
  peptide compound
WSGWSGCSVTCG

SEQ ID NO: 25 - protein, 12 aa, Artificial Sequence
  peptide compound
WSGWGSCSVTCG

SEQ ID NO: 26 - protein, 12 aa, Artificial Sequence
  peptide compound
WSGWGGCSVTCG

SEQ ID NO: 27 - protein, 12 aa, Artificial Sequence
  peptide compound
WSSWSSCSRTCG

SEQ ID NO: 28 - protein, 12 aa, artificial sequence
  peptide compound
WSSWSGCSRTCG

SEQ ID NO: 29 - protein, 12 aa, Artificial Sequence
  peptide compound
WSSWGSCSRTCG

SEQ ID NO: 30 - protein, 12 aa, Artificial Sequence
  peptide compound
WSSWGGCSRTCG

SEQ ID NO: 31 - protein, 12 aa, Artificial Sequence
  peptide compound
WSGWSSCSRTCG

SEQ ID NO: 32 - protein, 12 aa, Artificial Sequence
  peptide compound
WSGWSGCSRTCG

SEQ ID NO: 33 - protein, 12 aa, Artificial Sequence
  peptide compound
WSGWGSCSRTCG

SEQ ID NO: 34 - protein, 12 aa, Artificial Sequence
  peptide compound
WSGWGGCSRTCG

SEQ ID NO: 35 - protein, 13 aa, Artificial Sequence
  peptide compound
PWSGWSSCSRSCG

SEQ ID NO: 36 - protein, 14 aa, Artificial Sequence
  peptide compound
APWSGWSSCSRSCG

SEQ ID NO: 37 - protein, 15 aa, Artificial Sequence
  peptide compound
LAPWSGWSSCSRSCG

SEQ ID NO: 38 - protein, 16 aa, Artificial Sequence
  peptide compound
VLAPWSGWSSCSRSCG

SEQ ID NO: 39 - protein, 13 aa, Artificial Sequence
  peptide compound
WSGWSSCSRSCGL

SEQ ID NO: 40 - protein, 14 aa, Artificial Sequence
  peptide compound
WSGWSSCSRSCGLG

SEQ ID NO: 41 - protein, 15 aa, Artificial Sequence
  peptide compound
WSGWSSCSRSCGLGL

SEQ ID NO: 42 - protein, 16 aa, Artificial Sequence
  peptide compound
WSGWSSCSRSCGLGLI

SEQ ID NO: 43 - protein, 17 aa, Artificial Sequence
  peptide compound
WSGWSSCSRSCGLGLIF

SEQ ID NO: 44 - protein, 14 aa, Artificial Sequence
  peptide compound
PWSGWSSCSRSCGL

SEQ ID NO: 45 - protein, 15 aa, Artificial Sequence
  peptide compound
PWSGWSSCSRSCGLG

SEQ ID NO: 46 - protein, 16 aa, Artificial Sequence
  peptide compound
PWSGWSSCSRSCGLGL

SEQ ID NO: 47 - protein, 17 aa, Artificial Sequence
  peptide compound
PWSGWSSCSRSCGLGLI

SEQ ID NO: 48 - protein, 18 aa, Artificial Sequence
  peptide compound
PWSGWSSCSRSCGLGLIF

SEQ ID NO: 49 - protein, 15 aa, Artificial Sequence
  peptide compound
APWSGWSSCSRSCGL

SEQ ID NO: 50 - protein, 16 aa, Artificial Sequence
  peptide compound
APWSGWSSCSRSCGLG

SEQ ID NO: 51 - protein, 17 aa, Artificial Sequence
  peptide compound
APWSGWSSCSRSCGLGL

SEQ ID NO: 52 - protein, 18 aa, Artificial Sequence
  peptide compound
APWSGWSSCSRSCGLGLI

SEQ ID NO: 53 - protein, 19 aa, Artificial Sequence
  peptide compound
APWSGWSSCSRSCGLGLIF

SEQ ID NO: 54 - protein, 16 aa, Artificial Sequence
  peptide compound
LAPWSGWSSCSRSCGL

SEQ ID NO: 55 - protein, 17 aa, Artificial Sequence
  peptide compound
LAPWSGWSSCSRSCGLG

SEQ ID NO: 56 - protein, 18 aa, Artificial Sequence
  peptide compound
LAPWSGWSSCSRSCGLGL

SEQ ID NO: 57 - protein, 19 aa, Artificial Sequence
  peptide compound
LAPWSGWSSCSRSCGLGLI

SEQ ID NO: 58 - protein, 20 aa, Artificial Sequence
  peptide compound
LAPWSGWSSCSRSCGLGLIF

SEQ ID NO: 59 - protein, 17 aa, Artificial Sequence
  peptide compound
VLAPWSGWSSCSRSCGL

SEQ ID NO: 60 - protein, 18 aa, Artificial Sequence
  peptide compound
VLAPWSGWSSCSRSCGLG

SEQ ID NO: 61 - protein, 19 aa, Artificial Sequence
  peptide compound
VLAPWSGWSSCSRSCGLGL

SEQ ID NO: 62 - protein, 20 aa, Artificial Sequence
  peptide compound
VLAPWSGWSSCSRSCGLGLI

SEQ ID NO: 63 - protein, 21 aa, Artificial Sequence
  peptide compound
VLAPWSGWSSCSRSCGLGLIF